European Patent Application EP 4 273 246 A1, published November 8, 2023. Title: Recombinant Strain with Modified Gene BBD29_14900, and Method for Constructing the Same and Use Thereof. Applicant: NINGXIA EPPEN BIOTECH CO., LTD. The sequence listing filed with the application follows.

SEQUENCE LISTING (32 sequences)

SEQ ID NO: 1 - DNA, 1179 bp, Corynebacterium glutamicum
atgaccatcgacctgcagcgttccacccaaaacctcacccatgaggaaatcttcgaggcacacgagggcggaaagctctccattagttccactcgtccgctccgcgacatgcgcgatctttcccttgcttacaccccaggtgttgctcaggtttgtgaagcaatcaaagaagatccagaggttgcacgcacccacacgggcattggaaacaccgtcgcggttatttccgacggcaccgctgttcttggccttggcgatatcggacctcaggcatcccttcccgtcatggagggcaaggctcagctgttcagctctttcgctggtttgaaggctatccctatcgttttggatgttcacgatgttgacgctttggttgagaccatcgcagccatcgcgccttctttcggtgctatcaacttggaggacatctccgctcctcgttgcttcgaggtggagcgccgcctcatcgagcgtctcgatattccagttatgcacgatgaccagcacggcaccgctgtggttatcctcgctgcgctgcgcaactccctgaagctgctggatcgcaagatcgaagacctcaagattgttatttccggcgcaggcgcagcgggcgttgcagctgtagatatgttgaccaatgctggcgcaaccgacatcgtggttcttgattcccgaggcatcatccacgacagccgtgaggatctttccccagttaaggctgctctcgcggagaagaccaaccctcgtggcatcagcggtggcatcaatgaggctttcaccggcgcggacctgttcatcggcgtgtccggcggcaacatcggcgaggacgctctcaaactcatggcaccacagccaatcctgttcaccctggcgaacccaaccccagagatcgatcctgaactgtctcagaagtacggcgccatcgtcgcgaccggccgctctgacctgcctaaccagatcaacaacgtgctagcgttcccaggcattttcgccggcgctctcgcagccaaggccaagaagatcacccccgagatgaagctcgctgcagcagaggcaatcgccgacatcgcagctgaggacctcgaggtcggccgcatcgtaccgaccgccttggatccccgcgtcgccccagcagtaaaggcagctgtccaggccgtcgccgaagcgcaaaacgcttag

SEQ ID NO: 2 - DNA, 1179 bp, Artificial Sequence
  CDS
atgaccatcgacctgcagcgttccacccaaaacctcacccatgaggaaatcttcgaggcacacgagggcggaaagctctccattagttccactcgtccgctccgcgacatgcgcgatctttcccttgcttacaccccaggtgttgctcaggtttgtgaagcaatcaaagaagatccagaggttgcacgcacccacacgggcattggaaacaccgtcgcggttatttccgacggcaccgctgttcttggccttggcgatatcggacctcaggcatcccttcccgtcatggagggcaaggctcagctgttcagctctttcgctggtttgaaggctatccctatcgttttggatgttcacgatgttgacgctttggttgagaccatcgcagccatcgcgccttctttcggtgctatcaacttggaggacatctccgctcctcgttgcttcgaggtggagcgccgcctcatcgagcgtctcgatattccagttatgcacgatgaccagcacggcaccgctgtggttatcctcgctgcgctgcgcaactccctgaagctgctggatcgcaagatcgaagacctcaagattgttatttccggcgcaggcgcagcgggcgttgcagctgtagatatgttgaccaatgctggcgcaaccgacatcgtggttcttgattcccgaggcatcatccacgacagccgtgaggatctttccccagttaaggctgctctcgcggagaagaccaaccctcgtggcatcagcggtggcatcaatgaggctttcaccggcgcggacctgttcatcggcgtgtccggcggcaacatcggcgaggacgctctcaaactcatggcaccacagccaatcctgttcaccctggcgaacccaaccccagagatcgatcctgaactgtctcagaagtacggcgccatcgtcgcgaccggccgctctgacctgcctaaccagatcaacaacgtgctagcgttcccaggcattttcgccggcgctctcgcagccaaggccaagaagatcacccccgagatgaagctcgctgcagcagaggcaatcgccgacatcgcagctgaggacctcgaggtcggccgcatcgtaccgaccgccttgaatccccgcgtcgccccagcagtaaaggcagctgtccaggccgtcgccgaagcgcaaaacgcttag

SEQ ID NO: 3 - protein, 392 aa, Corynebacterium glutamicum
MTIDLQRSTQNLTHEEIFEAHEGGKLSISSTRPLRDMRDLSLAYTPGVAQVCEAIKEDPEVARTHTGIGNTVAVISDGTAVLGLGDIGPQASLPVMEGKAQLFSSFAGLKAIPIVLDVHDVDALVETIAAIAPSFGAINLEDISAPRCFEVERRLIERLDIPVMHDDQHGTAVVILAALRNSLKLLDRKIEDLKIVISGAGAAGVAAVDMLTNAGATDIVVLDSRGIIHDSREDLSPVKAALAEKTNPRGISGGINEAFTGADLFIGVSGGNIGEDALKLMAPQPILFTLANPTPEIDPELSQKYGAIVATGRSDLPNQINNVLAFPGIFAGALAAKAKKITPEMKLAAAEAIADIAAEDLEVGRIVPTALDPRVAPAVKAAVQAVAEAQNA

SEQ ID NO: 4 - protein, 392 aa, Artificial Sequence
  Glutamate synthesis
MTIDLQRSTQNLTHEEIFEAHEGGKLSISSTRPLRDMRDLSLAYTPGVAQVCEAIKEDPEVARTHTGIGNTVAVISDGTAVLGLGDIGPQASLPVMEGKAQLFSSFAGLKAIPIVLDVHDVDALVETIAAIAPSFGAINLEDISAPRCFEVERRLIERLDIPVMHDDQHGTAVVILAALRNSLKLLDRKIEDLKIVISGAGAAGVAAVDMLTNAGATDIVVLDSRGIIHDSREDLSPVKAALAEKTNPRGISGGINEAFTGADLFIGVSGGNIGEDALKLMAPQPILFTLANPTPEIDPELSQKYGAIVATGRSDLPNQINNVLAFPGIFAGALAAKAKKITPEMKLAAAEAIADIAAEDLEVGRIVPTALNPRVAPAVKAAVQAVAEAQNA

SEQ ID NO: 5 - DNA, 56 bp, Artificial Sequence
  primer
cagtgccaagcttgcatgcctgcaggtcgactctagcgctgtggttatcctcgctg

SEQ ID NO: 6 - DNA, 30 bp, Artificial Sequence
  primer
ctggggcgacgcggggattcaaggcggtcg

SEQ ID NO: 7 - DNA, 30 bp, Artificial Sequence
  primer
cgaccgccttgaatccccgcgtcgccccag

SEQ ID NO: 8 - DNA, 58 bp, Artificial Sequence
  primer
cagctatgaccatgattacgaattcgagctcggtaccctgagtgtcactaggctagtc

SEQ ID NO: 9 - DNA, 20 bp, Artificial Sequence
  primer
gcagccaaggccaagaagat

SEQ ID NO: 10 - DNA, 20 bp, Artificial Sequence
  primer
tccctgtttaagactgcatt

SEQ ID NO: 11 - DNA, 56 bp, Artificial Sequence
  primer
cagtgccaagcttgcatgcctgcaggtcgactctaggacccgcttgccatacgaag

SEQ ID NO: 12 - DNA, 40 bp, Artificial Sequence
  primer
agtgggctgaatttgggctgatctactcatctgaagaatc

SEQ ID NO: 13 - DNA, 40 bp, Artificial Sequence
  primer
gattcttcagatgagtagatcagcccaaattcagcccact

SEQ ID NO: 14 - DNA, 40 bp, Artificial Sequence
  primer
caaaccagagtgcccacgaactaagcgttttgcgcttcgg

SEQ ID NO: 15 - DNA, 40 bp, Artificial Sequence
  primer
ccgaagcgcaaaacgcttagttcgtgggcactctggtttg

SEQ ID NO: 16 - DNA, 58 bp, Artificial Sequence
  primer
cagctatgaccatgattacgaattcgagctcggtaccccataagaaacaaccacttcc

SEQ ID NO: 17 - DNA, 20 bp, Artificial Sequence
  primer
gtccaaggtgacggccgcac

SEQ ID NO: 18 - DNA, 20 bp, Artificial Sequence
  primer
gcagccttaactggggaaag

SEQ ID NO: 19 - DNA, 20 bp, Artificial Sequence
  primer
ggagcgccgcctcatcgagc

SEQ ID NO: 20 - DNA, 20 bp, Artificial Sequence
  primer
atattcggcccagcagcagc

SEQ ID NO: 21 - DNA, 56 bp, Artificial Sequence
  primer
gcttgcatgcctgcaggtcgactctagaggatcccccagcccaaattcagcccact

SEQ ID NO: 22 - DNA, 54 bp, Artificial Sequence
  primer
atcaggctgaaaatcttctctcatccgccaaaacctaagcgttttgcgcttcgg

SEQ ID NO: 23 - DNA, 56 bp, Artificial Sequence
  primer
cagtgccaagcttgcatgcctgcaggtcgactctagtcgctgaaacagcaggggac

SEQ ID NO: 24 - DNA, 40 bp, Artificial Sequence
  primer
aggcgtcgataagcaaatttatcatttagccttgttaatc

SEQ ID NO: 25 - DNA, 40 bp, Artificial Sequence
  primer
gattaacaaggctaaatgataaatttgcttatcgacgcct

SEQ ID NO: 26 - DNA, 58 bp, Artificial Sequence
  primer
cagctatgaccatgattacgaattcgagctcggtacccaacttgccatgagtcgtctt

SEQ ID NO: 27 - DNA, 20 bp, Artificial Sequence
  primer
tcgctgaaacagcaggggac

SEQ ID NO: 28 - DNA, 20 bp, Artificial Sequence
  primer
aacttgccatgagtcgtctt

SEQ ID NO: 29 - DNA, 1253 bp, Artificial Sequence
  Coding sequence
cagtgccaagcttgcatgcctgcaggtcgactctagcgctgtggttatcctcgctgcgctgcgcaactccctgaagctgctggatcgcaagatcgaagacctcaagattgttatttccggcgcaggcgcagcgggcgttgcagctgtagatatgttgaccaatgctggcgcaaccgacatcgtggttcttgattcccgaggcatcatccacgacagccgtgaggatctttccccagttaaggctgctctcgcggagaagaccaaccctcgtggcatcagcggtggcatcaatgaggctttcaccggcgcggacctgttcatcggcgtgtccggcggcaacatcggcgaggacgctctcaaactcatggcaccacagccaatcctgttcaccctggcgaacccaaccccagagatcgatcctgaactgtctcagaagtacggcgccatcgtcgcgaccggccgctctgacctgcctaaccagatcaacaacgtgctagcgttcccaggcattttcgccggcgctctcgcagccaaggccaagaagatcacccccgagatgaagctcgctgcagcagaggcaatcgccgacatcgcagctgaggacctcgaggtcggccgcatcgtaccgaccgccttgaatccccgcgtcgccccagcagtaaaggcagctgtccaggccgtcgccgaagcgcaaaacgcttagaaatttgcttatcgacgcctccctccccgatagcgaacctccaagccctatcagtctctgatggggcttgggggttcgcaccatgtttatcgaaatgcagtcttaaacagggaatgacataatcaggcctatgagcgcccctgacattactgctgcagacctaaaagtttttgaaaactcggggataacggaccattcgacaatcttattaggcgcaggcgcttccattacgtcgggtctacctgactggaatactcttgccgtaagtttgcttctgcgcagtaacgccgtcaaacaagaagaagttgcagagcttctgctgaatcatcaagatcctatgatcgttgtcgaatccgcaaaagttgaaagcggtgaatcgtgggacgttttgctgaaagaatgcctttacgctgactctgttccagtggctgaactcatcccgtcggctttacatcgcgcggttgtagggcactttctcgctaaacctgacaagactagcctagtgacactcagggtaccgagctcgaattcgtaatcatggtcatagctg

SEQ ID NO: 30 - DNA, 3008 bp, Artificial Sequence
  Homologous arm
cagtgccaagcttgcatgcctgcaggtcgactctaggacccgcttgccatacgaagtcctggagaagatctccacccgcatcaccaacgaagttccagacgtaaaccgcgtggttttggacgtaacctccaagccaccaggaaccatcgaatgggagtaggccttaaatgagccttcgttaagcggcaatcaccttatcggtgattgccgctttcccatttctccgggttttctggaactttttgggcgtatgctgggaatgatcttattattttgatttcagaaagcaggagagaccagatgagcgaaatccttgaaacctactgggcaccccacttcggaaacaccgatgaagccgcagcactcgtttcatacttggcacaagcttccggtgatcctattgaggttcacaccctgttcggggatttaggtttagacggactctctggaaactacaccgacactgagatcgacggctacggcgacgcattcctgctggttgcagcactagcagtgttgatggctgaaaacaaagcatccggcggcgtgaatctgggtgaagttgggggagctgataaatcgatccggctgcatgttgaatccaaggaaaacacccagatcaacaccgcattgaagtactttgcgctttccccagaagaccacgcagcggcagatcgcttcgatgaggatgacctgtctgagcttgccaacttgagtgaagagctgcgcggacagctggactaattgctgcccgtttaaggagtccgattcttcagatgagtagatcagcccaaattcagcccactgaatcaaccactgaatcaaccactgaatcaaccccaaaaccacccaaaagtcacacttagcaaacaattaaattcatcacaaaacacccctgcacaaacttagcaataaaggtcaggggtgttttgcaaatgttcacattgcgaattttttgttgagctacagatttagctagtgtttttgttccagaaccctaaatgaggttctacccttaacagagcttcccgcaaaaacaccgattaacaaggctaaatgatatgaccatcgacctgcagcgttccacccaaaacctcacccatgaggaaatcttcgaggcacacgagggcggaaagctctccattagttccactcgtccgctccgcgacatgcgcgatctttcccttgcttacaccccaggtgttgctcaggtttgtgaagcaatcaaagaagatccagaggttgcacgcacccacacgggcattggaaacaccgtcgcggttatttccgacggcaccgctgttcttggccttggcgatatcggacctcaggcatcccttcccgtcatggagggcaaggctcagctgttcagctctttcgctggtttgaaggctatccctatcgttttggatgttcacgatgttgacgctttggttgagaccatcgcagccatcgcgccttctttcggtgctatcaacttggaggacatctccgctcctcgttgcttcgaggtggagcgccgcctcatcgagcgtctcgatattccagttatgcacgatgaccagcacggcaccgctgtggttatcctcgctgcgctgcgcaactccctgaagctgctggatcgcaagatcgaagacctcaagattgttatttccggcgcaggcgcagcgggcgttgcagctgtagatatgttgaccaatgctggcgcaaccgacatcgtggttcttgattcccgaggcatcatccacgacagccgtgaggatctttccccagttaaggctgctctcgcggagaagaccaaccctcgtggcatcagcggtggcatcaatgaggctttcaccggcgcggacctgttcatcggcgtgtccggcggcaacatcggcgaggacgctctcaaactcatggcaccacagccaatcctgttcaccctggcgaacccaaccccagagatcgatcctgaactgtctcagaagtacggcgccatcgtcgcgaccggccgctctgacctgcctaaccagatcaacaacgtgctagcgttcccaggcattttcgccggcgctctcgcagccaaggccaagaagatcacccccgagatgaagctcgctgcagcagaggcaatcgccgacatcgcagctgaggacctcgaggtcggccgcatcgtaccgaccgccttgaatccccgcgtcgccccagcagtaaaggcagctgtccaggccgtcgccgaagcgcaaaacgcttagttcgtgggcactctggtttggttaccaggatgggttagtcattctgatcagcgaattccacgttcacatcgccaattccagagttcacaaccagattcagcattggaccttctagatcagcattgtgggcggtgagatctccaacatcacagcgcgctgtgcccacaccggcggtacaacttaggctcacgggcacatcatcgggcagggtgaccatgacttcgccgatccctgaggtgatttggatgttttgttcctgatccaattgggtgaggtggctgaaatcgaggttcatttcacccacgccagaggtgtagctgctgaggagttcatcgttggtggggatgagattgacatcgccgattccagggtcgtcttcaaagtagatgggatcgatatttgaaataaacaggcctgcgagggcgctcatgacaactccggtaccaactacaccgccgacaatccatggccacacatggcgctttttctgaggcttttgtggagggacttgtacatcccaggtgttgtattggttttgggcaagtggatcccaatgaggcgcttcgggggtttgttgcgcgaagggtgcatagtagccctcaacgggggtgatagtgcttagatctggttggggttgtgggtagagatcttcgtttttcatggtggcatcctcagaaacagtgaattcagtggtgagtagtccgcggggtggaagtggttgtttcttatggggtaccgagctcgaattcgtaatcatggtcatagctg

SEQ ID NO: 31 - DNA, 1524 bp, Artificial Sequence
  Coding sequence
gcttgcatgcctgcaggtcgactctagaggatcccccagcccaaattcagcccactgaatcaaccactgaatcaaccactgaatcaaccccaaaaccacccaaaagtcacacttagcaaacaattaaattcatcacaaaacacccctgcacaaacttagcaataaaggtcaggggtgttttgcaaatgttcacattgcgaattttttgttgagctacagatttagctagtgtttttgttccagaaccctaaatgaggttctacccttaacagagcttcccgcaaaaacaccgattaacaaggctaaatgatatgaccatcgacctgcagcgttccacccaaaacctcacccatgaggaaatcttcgaggcacacgagggcggaaagctctccattagttccactcgtccgctccgcgacatgcgcgatctttcccttgcttacaccccaggtgttgctcaggtttgtgaagcaatcaaagaagatccagaggttgcacgcacccacacgggcattggaaacaccgtcgcggttatttccgacggcaccgctgttcttggccttggcgatatcggacctcaggcatcccttcccgtcatggagggcaaggctcagctgttcagctctttcgctggtttgaaggctatccctatcgttttggatgttcacgatgttgacgctttggttgagaccatcgcagccatcgcgccttctttcggtgctatcaacttggaggacatctccgctcctcgttgcttcgaggtggagcgccgcctcatcgagcgtctcgatattccagttatgcacgatgaccagcacggcaccgctgtggttatcctcgctgcgctgcgcaactccctgaagctgctggatcgcaagatcgaagacctcaagattgttatttccggcgcaggcgcagcgggcgttgcagctgtagatatgttgaccaatgctggcgcaaccgacatcgtggttcttgattcccgaggcatcatccacgacagccgtgaggatctttccccagttaaggctgctctcgcggagaagaccaaccctcgtggcatcagcggtggcatcaatgaggctttcaccggcgcggacctgttcatcggcgtgtccggcggcaacatcggcgaggacgctctcaaactcatggcaccacagccaatcctgttcaccctggcgaacccaaccccagagatcgatcctgaactgtctcagaagtacggcgccatcgtcgcgaccggccgctctgacctgcctaaccagatcaacaacgtgctagcgttcccaggcattttcgccggcgctctcgcagccaaggccaagaagatcacccccgagatgaagctcgctgcagcagaggcaatcgccgacatcgcagctgaggacctcgaggtcggccgcatcgtaccgaccgccttgaatccccgcgtcgccccagcagtaaaggcagctgtccaggccgtcgccgaagcgcaaaacgcttaggttttggcggatgagagaagattttcagcctgat

SEQ ID NO: 32 - DNA, 1555 bp, Artificial Sequence
  Homologous arm
cagtgccaagcttgcatgcctgcaggtcgactctagtcgctgaaacagcaggggacagcttcgtgtccattggcttgttcgccttcggtgcactcggactcattggcgtgacagtggcaacccgaactgtggatcaacgcatgctgcgtggaagtgttcacaccaccactttgtttgtcattgctgcaattctcggacagatcgcattcggattagagggcacactagccgtagtagctatcttccttgcagtcaccgtgtttggtggagcatacggcgctctcccaaccctgggaaccaccatcttcctccatgcgggtcgcgaccacccagatactgcatcctccatttatgtggtcacttaccaagtgggtatcgcgtctggcgcggcacttggcgcgatggctgtggatgccgattgggttgctggcactttgtggatcatggctggactgtcattggcttccacgttggtcttggcgctgtggtcccgcccgctactgaagtagcagcccaaattcagcccactgaatcaaccactgaatcaaccactgaatcaaccccaaaaccacccaaaagtcacacttagcaaacaattaaattcatcacaaaacacccctgcacaaacttagcaataaaggtcaggggtgttttgcaaatgttcacattgcgaattttttgttgagctacagatttagctagtgtttttgttccagaaccctaaatgaggttctacccttaacagagcttcccgcaaaaacaccgattaacaaggctaaatgataaatttgcttatcgacgcctccctccccgatagcgaacctccaagccctatcagtctctgatggggcttgggggttcgcaccatgtttatcgaaatgcagtcttaaacagggaatgacataatcaggcctatgagcgcccctgacattactgctgcagacctaaaagtttttgaaaactcggggataacggaccattcgacaatcttattaggcgcaggcgcttccattacgtcgggtctacctgactggaatactcttgccgtaagtttgcttctgcgcagtaacgccgtcaaacaagaagaagttgcagagcttctgctgaatcatcaagatcctatgatcgttgtcgaatccgcaaaagttgaaagcggtgaatcgtgggacgttttgctgaaagaatgcctttacgctgactctgttccagtggctgaactcatcccgtcggctttacatcgcgcggttgtagggcactttctcgctaaacctgacaagactagcctagtgacactcaattttgatgcgatcttagaacttgctctagaaaatgagcttgaaggcgctataaaagtcgagtcgattacgtccggagcccagacggagaaaattgatgctacgcaggtcatagaagttcatcatttacatggaatcatcaccccggattatgccaatgatgtgatacttacttttacagattttgcacaactgattgagcaagacgactcatggcaagttgggtaccgagctcgaattcgtaatcatggtcatagctg